European Patent Specification EP 3 866 860 B1, published January 8, 2025. Title: Complement Component 1s (C1s) Deficient Cells for Production Of Vaccines and Biopharmaceutical Proteins. Applicant: THE REGENTS OF THE UNIVERSITY OF CALIFORNIA. Application EP19873893.2. The sequence listing filed with the application follows.

SEQUENCE LISTING (58 sequences)

SEQ ID NO: 1 - protein, 472 aa, Artificial sequence
  synthetic sequence
VPVWKEADTTLFCASDAKAHETEVHNVWATHACVPTDPNPQEIDLENVTENFNMWKNNMVEQMQEDVISLWDQSLKPCVKLTPPCVTLHCTNANLTKANLTNVNNRTNVSNIIGNITDEVRNCSFNMTTELRDKKQKVHALFYKLDIVPIEDNNDSSEYRLINCNTSVIKQACPKISFDPIPIHYCTPAGYAILKCNDKNFNGTGPCKNVSSVQCTHGIKPVVSTQLLLNGSLAEEEIIIRSENLTNNAKTIIVHLNKSVVINCTRPSNNTRTSITIGPGQVFYRTGDIIGDIRKAYCNISGTEWNKALKQVTEKLKEHFNNKPIIFQPPSGGDLEITMHHFNCRGEFFYCNTTRLFNNTCIANGTIEGCNGNITLPCKIKQIINMWQGAGQAMYAPPISGTINCVSNITGILLTRDGGATNNTNNETFRPGGGNIKDNWRNELYKYKVVQIEPLGVAPTRAKRRVVEREKR

SEQ ID NO: 2 - protein, 462 aa, Artificial sequence
  synthetic sequence
VPVWKEADTTLFCASDAKAHETEVHNVWATHACVPTDPNPQEIDLENVTENFNMWKNNMVEQMQEDVISLWDQSLKPCVKLTPPCVTLHCTNANLTKANLTNVNNRTNVSNIIGNITDEVRNCSFNMTTELRDKKQKVHALFYKLDIVPIEDNNDSSEYRLINCNTSVIKQACPKISFDPIPIHYCTPAGYAILKCNDKNFNGTGPCKNVSSVQCTHGIKPVVSTQLLLNGSLAEEEIIIRSENLTNNAKTIIVHLNKSVVINCTRPSNNTRTSITIGPGQVFYRTGDIIGDIRKAYCNISGTEWNKALKQVTEKLKEHFNNKPIIFQPPSGGDLEITMHHFNCRGEFFYCNTTRLFNNTCIANGTIEGCNGNITLPCKIKQIINMWQGAGQAMYAPPISGTINCVSNITGILLTRDGGATNNTNNETFRPGGGNIKDNWRNELYKYKVVQIEPLGVAPTRA

SEQ ID NO: 3 - protein, 517 aa, Artificial sequence
  synthetic sequence
MGGAAARLGAVILFVVIVGLHGVRGKYALADASLKMADPNRFRGKDLPVLDQLLEVPVWKEADTTLFCASDAKAHETEVHNVWATHACVPTDPNPQEIDLENVTENFNMWKNNMVEQMQEDVISLWDQSLKPCVKLTPPCVTLHCTNANLTKANLTNVNNRTNVSNIIGNITDEVRNCSFNMTTELRDKKQKVHALFYKLDIVPIEDNNDSSEYRLINCNTSVIKQACPKISFDPIPIHYCTPAGYAILKCNDKNFNGTGPCKNVSSVQCTHGIKPVVSTQLLLNGSLAEEEIIIRSENLTNNAKTIIVHLNKSVVINCTRPSNNTRTSITIGPGQVFYRTGDIIGDIRKAYCNISGTEWNKALKQVTEKLKEHFNNKPIIFQPPSGGDLEITMHHFNCRGEFFYCNTTRLFNNTCIANGTIEGCNGNITLPCKIKQIINMWQGAGQAMYAPPISGTINCVSNITGILLTRDGGATNNTNNETFRPGGGNIKDNWRNELYKYKVVQIEPLGVAPTRA

SEQ ID NO: 4 - DNA, 2088 bp, Cricetulus griseus
atgggcaaatcaccagaggcatggtgcattgtcttgttttctgttttggcatcattttctgccgagcctaccatgcatggggagatcctgtcccctaactatcctcaggcgtaccccaatgagatcgagaaaacgtgggacatagaagtcccagaagggtttgggattcgcctctacttcacccatctggacatggagctgtcagagaactgcgaatatgactcggtgcagataatctcaggaggcgtcgaggaagggagactctgtgggcagaggaccagcaagaatgccaactcccccattgtggaagagtttcaaatgccatacaataaactccaggtgatctttaggtcagacttctccaacgaagagcggtttactggctttgctgcatattacgctgccgtagatataaatgaatgcacagattttacagatgtcccttgcagccacttctgcaataatttcattggtggttacttctgctcctgtcccccagaatacttcctccacgatgacatgaggaactgcggagtcaattgtagtgggaatgtattcactgccctgattggggagatttcaagccccaattatcccagtccataccccgagaactcaaggtgtgaataccagattttgctggaggaggggttccaagtggtggtgactatccggagagaagattttgatgtggaaccagctgactcggaggggaactgccaggacagtttactctttgctgcaaaaaatcaactatttggtccttactgtggcaatgggttccctgggccactaactattgaaacccacagtaacactcttgacattgtctttcaaacggacctaacagagcaaagaaaaggctggaagcttcgttaccatggagacccaatcccttgtcccaaggaaatcactgccaattctgtttgggtgcctgaaaaggcaaaatatgtgtttaaagatgtggtgaagatatcctgtgtggacggatttgaagttgtagagggaaatgttggctcagcattcttctattctacttgtcaaagcaatggacagtggagtaattccagactacaatgtcagcctgtggactgtggtattccggaacccattcagaatggtaaagttgacgatccagaaaacactgtgtttggctctgtcatccagtactcgtgcgaggagccatattactacatggaacatgaagaacacggcggggagtatcgctgcgctgctaatgggagctgggtgaatgacgaactgggcatagagctcccaaaatgtgttccagtctgtggggtacccactgagcccattgcattacagcagaggatatttggaggattccctgcaaagatccagagttttccttggcaagtcttctttgagtccccacgggccggtggggctcttattgacgagtactgggtgttgacagccgctcatgttgtggagggaaactctgacccatctatgtatgtggggaccacatttgtgagaatggaacatctggcgaatgcccagaggctcaccgctgaacgtgtgattattcatccaggctggaagccagcggatgacctagaaacacggacaaattttgacaatgacattgcactggtgcagctgaaagaccccgtgaaaatggggcccactgtctcccccatctgcctgccaggtacctcctcagagtacaacccctcaaagaatgacctgggactgatctcagggtggggccgaacagagaagagaaatattgttccccaactcaaaggggcaaagttacctgtgacctctttagagaagtgccaacaggtgaaaggggagaactccaaagtgagggcggatgactacgttttcaccagcaacatgatctgtgctggagagaaaggtgttgatagctgtcagggggacagtggtggggcttttgctttgcaggtccccaatgtaaaggaccccaaattctatgtggcaggcctagtgtcctgggggaaaaagtgtgggacctatggaatctacacaaaggtaaagaactacatggattggatcgtgaagacgatgcaggagaatagtgtccccagtaaggactaa

SEQ ID NO: 5 - protein, 684 aa, Cricetulus griseus
MRVKETQMNWPNLWKWGTLILGLVIICSASDNLWVTVYYGVPVWKEADTTLFCASDAKAHETEVHNVWATHACVPTDPNPQEIDLENVTENFNMWKNNMVEQMQEDVISLWDQSLKPCVKLTPLCVTLHCTNANLTKANLTNVNNRTNVSNIIGNITDEVRNCSFNMTTELRDKKQKVHALFYKLDIVPIEDNNDSSEYRLINCNTSVIKQACPKISFDPIPIHYCTPAGYAILKCNDKNFNGTGPCKNVSSVQCTHGIKPVVSTQLLLNGSLAEEEIIIRSDNLTNNAKTIIVHLNKSVVINCTRPSNNTRTSITIGPGQVFYRTGDIIGDIRKAYCEINGTEWNKALKQVTEKLKEHFNNKPIIFQPPSGGDLEITMHHFNCRGEFFYCNTTRLFNNTCIANGTIEGCNGNITLPCKIKQIINMWQGAGQAMYAPPISGTINCVSNITGILLTRDGGATNNTNNETFRPGGGNIKDNWRNELYKYKVVQIEPLGVAPTRAKRRVVEREKRAVGIGAMIFGFLGAAGSTMGAASITLTVQARQLLSGIVQQQSNLLRAIEAQQHLLQLTVWGIKQLQARVLAVERYLKDQKFLGLWGCSGKIICTTAVPWNSTWSNKSLEEIWSNMTWIEWEREISNYTNQIYEILTKSQDQQDRNEKDLLELDKWASLWTWFDITNWLWYIK

SEQ ID NO: 6 - protein, 695 aa, Artificial sequence
  synthetic sequence
MGKSPEAWCIVLFSVLASFSAEPTMHGEILSPNYPQAYPNEIEKTWDIEVPEGFGIRLYFTHLDMELSENCEYDSVQIISGGVEEGRLCGQRTSKNANSPIVEEFQMPYNKLQVIFRSDFSNEERFTGFAAYYAAVDINECTDFTDVPCSHFCNNFIGGYFCSCPPEYFLHDDMRNCGVNCSGNVFTALIGEISSPNYPSPYPENSRCEYQILLEEGFQVVVTIRREDFDVEPADSEGNCQDSLLFAAKNQLFGPYCGNGFPGPLTIETHSNTLDIVFQTDLTEQRKGWKLRYHGDPIPCPKEITANSVWVPEKAKYVFKDVVKISCVDGFEVVEGNVGSAFFYSTCQSNGQWSNSRLQCQPVDCGIPEPIQNGKVDDPENTVFGSVIQYSCEEPYYYMEHEEHGGEYRCAANGSWVNDELGIELPKCVPVCGVPTEPIALQQRIFGGFPAKIQSFPWQVFFESPRAGGALIDEYWVLTAAHVVEGNSDPSMYVGTTFVRMEHLANAQRLTAERVIIHPGWKPADDLETRTNFDNDIALVQLKDPVKMGPTVSPICLPGTSSEYNPSKNDLGLISGWGRTEKRNIVPQLKGAKLPVTSLEKCQQVKGENSKVRADDYVFTSNMICAGEKGVDSCQGDSGGAFALQVPNVKDPKFYVAGLVSWGKKCGTYGIYTKVKNYMDWIVKTMQENSVPSKD

SEQ ID NO: 7 - protein, 684 aa, Artificial sequence
  synthetic sequence
MRVKETQMNWPNLWKWGTLILGLVIICSASDNLWVTVYYGVPVWKEADTTLFCASDAKAHETEVHNVWATHACVPTDPNPQEIDLENVTENFNMWKNNMVEQMQEDVISLWDQSLKPCVKLTPLCVTLHCTNANLTKANLTNVNNRTNVSNIIGNITDEVRNCSFNMTTELRDKKQKVHALFYKLDIVPIEDNNDSSEYRLINCNTSVIKQACPKISFDPIPIHYCTPAGYAILKCNDKNFNGTGPCKNVSSVQCTHGIKPVVSTQLLLNGSLAEEEIIIRSDNLTNNAKTIIVHLNKSVVINCTRPSNNTRTSITIGPGQVFYRTGDIIGDIRKAYCNISGTEWNKALKQVTEKLKEHFNNKPIIFQPPSGGDLEITMHHFNCRGEFFYCNTTRLFNNTCIANGTIEGCNGNITLPCKIKQIINMWQGAGQAMYAPPISGTINCVSNITGILLTRDGGATNNTNNETFRPGGGNIKDNWRNELYKYKVVQIEPLGVAPTRAKRRVVEREKRAVGIGAMIFGFLGAAGSTMGAASITLTVQARQLLSGIVQQQSNLLRAIEAQQHLLQLTVWGIKQLQARVLAVERYLKDQKFLGLWGCSGKIICTTAVPWNSTWSNKSLEEIWSNMTWIEWEREISNYTNQIYEILTKSQDQQDRNEKDLLELDKWASLWTWFDITNWLWYIK

SEQ ID NO: 8 - DNA, 2084 bp, Artificial sequence
  synthetic sequence
atgggcaaatcaccagaggcatggtgcattgtcttgttttctgttttggcatcattttctgccgagcctaccatgcatggggagatcctgtcccctaactatcctcaggcgtaccccaatgagatcgagaaaacgtgggacatagaagtcccagaagggtttgggattcgcctctacttcacccatctggacatggagctgtcagagaactgcgaatatgactcggtgcagataatctcaggaggcgtcgaggaagggagactctgtgggcagaggaccagcaagaatgccaactcccccattgtggaagagtttcaaatgccatacaataaactccaggtgatctttaggtcagacttctccaacgaagagcggtttactggctttgctgcatattacgctgccgtagatataaatgaatgcacagattttacagatgtcccttgcagccacttctgcaataatttcattggtggttacttctgctcctgtcccccagaatacttcctccacgatgacatgaggaactgcggagtcaattgtagtgggaatgtattcactgccctgattggggagatttcaagccccaattatcccagtccataccccgagaactcaaggtgtgaataccagattttgctggaggaggggttccaagtggtggtgactatccggagagaagattttgatgtggaaccagctgactcggaggggaactgccaggacagtttactctttgctgcaaaaaatcaactatttggtccttactgtggcaatgggttccctgggccactaactattgaaacccacagtaacactcttgacattgtctttcaaacggacctaacagagcaaagaaaaggctggaagcttcgttaccatggagacccaatcccttgtcccaaggaaatcactgccaattctgtttgggtgcctgaaaaggcaaaatatgtgtttaaagatgtggtgaagatatcctgtgtggacggatttgaagttgtagagggaaatgttggctcagcattcttctattctacttgtcaaagcaatggacagtggagtaattccagactacaatgtcagcctgtggactgtggtattccggaacccattcagaatggtaaagttgacgatccagaaaacactgtgtttggctctgtcatccagtactcgtgcgaggagccatattactacatggaacatgaagaacacggcggggagtatcgctgcgctgctaatgggagctgggtgaatgacgaactgggcatagagctcccaaaatgtgttccagtctgtggggtacccactgagcccattgcattacagcagaggatatttggaggattccctgcaaagatccagagttttccttggcaagtcttctttgagtccccacgggccggtggggctcttattgacgagtactgggtgttgacagccgctcatgggagggaaactctgacccatctatgtatgtggggaccacatttgtgagaatggaacatctggcgaatgcccagaggctcaccgctgaacgtgtgattattcatccaggctggaagccagcggatgacctagaaacacggacaaattttgacaatgacattgcactggtgcagctgaaagaccccgtgaaaatggggcccactgtctcccccatctgcctgccaggtacctcctcagagtacaacccctcaaagaatgacctgggactgatctcagggtggggccgaacagagaagagaaatattgttccccaactcaaaggggcaaagttacctgtgacctctttagagaagtgccaacaggtgaaaggggagaactccaaagtgagggcggatgactacgttttcaccagcaacatgatctgtgctggagagaaaggtgttgatagctgtcagggggacagtggtggggcttttgctttgcaggtccccaatgtaaaggaccccaaattctatgtggcaggcctagtgtcctgggggaaaaagtgtgggacctatggaatctacacaaaggtaaagaactacatggattggatcgtgaagacgatgcaggagaatagtgtccccagtaaggactaa

SEQ ID NO: 9 - protein, 463 aa, Artificial sequence
  synthetic sequence
  misc_feature (191)..(191): Xaa can be any naturally occurring amino acid
VPVWKEATTTLFCASDAKAYDTEAHNVWATHACVPTDPNPQEVELVNVTENFNMWKNNMVEQMHEDIISLWDQSLKPCVKLTPLCVTLNCTDLRNTTNTNNSTDNNNSKSEGTIKGGEMKNCSFNITTSIGDKMQKEYALLYKLDIEPIDNDSTSYRLISCNTSVITQACPKISFEPIPIHYCAPAGFAIXKCNDKKFSGKGSCKNVSTVQCTHGIRPVVSTQLLLNGSLAEEEVVIRSEDFTDNAKTIIVHLNESVQINCTRPNNNTRKRIHIGPGRAFYTTKNIKGTIRQAHCNISRAKWNDTLRQIVSKLKEQFKNKTIVFNPSSGGDPEIVMHSFNCGGEFFYCNTSPLFNSIWNGNNTWNNTTGSNNNITLQCKIKQIINMWQKVGKAMYAPPIEGQIRCSSNITGLLLTRDGGEDTDTNDTEIFRPGGGDMRDNWRSELYKYKVVTIEPLGVAPTKA

SEQ ID NO: 10 - protein, 526 aa, Artificial sequence
  synthetic sequence
  misc_feature (246)..(246): Xaa can be any naturally occurring amino acid
MGGAAARLGAVILFVVIVGLHGVRGKYALADASLKMADPNRFRGKDLPVLDQLLEVPVWKEATTTLFCASDAKAYDTEAHNVWATHACVPTDPNPQEVELVNVTENFNMWKNNMVEQMHEDIISLWDQSLKPCVKLTPLCVTLNCTDLRNTTNTNNSTDNNNSKSEGTIKGGEMKNCSFNITTSIGDKMQKEYALLYKLDIEPIDNDSTSYRLISCNTSVITQACPKISFEPIPIHYCAPAGFAIXKCNDKKFSGKGSCKNVSTVQCTHGIRPVVSTQLLLNGSLAEEEVVIRSEDFTDNAKTIIVHLNESVQINCTRPNNNTRKRIHIGPGRAFYTTKNIKGTIRQAHCNISRAKWNDTLRQIVSKLKEQFKNKTIVFNPSSGGDPEIVMHSFNCGGEFFYCNTSPLFNSIWNGNNTWNNTTGSNNNITLQCKIKQIINMWQKVGKAMYAPPIEGQIRCSSNITGLLLTRDGGEDTDTNDTEIFRPGGGDMRDNWRSELYKYKVVTIEPLGVAPTKAKRRVVQRE

SEQ ID NO: 11 - protein, 497 aa, Artificial sequence
  synthetic sequence
MGKSPEAWCIVLFSVLASFSAEPTMHGEILSPNYPQAYPNEIEKTWDIEVPEGFGIRLYFTHLDMELSENCEYDSVQIISGGVEEGRLCGQRTSKNANSPIVEEFQMPYNKLQVIFRSDFSNEERFTGFAAYYAAVDINECTDFTDVPCSHFCNNFIGGYFCSCPPEYFLHDDMRNCGVNCSGNVFTALIGEISSPNYPSPYPENSRCEYQILLEEGFQVVVTIRREDFDVEPADSEGNCQDSLLFAAKNQLFGPYCGNGFPGPLTIETHSNTLDIVFQTDLTEQRKGWKLRYHGDPIPCPKEITANSVWVPEKAKYVFKDVVKISCVDGFEVVEGNVGSAFFYSTCQSNGQWSNSRLQCQPVDCGIPEPIQNGKVDDPENTVFGSVIQYSCEEPYYYMEHEEHGGEYRCAANGSWVNDELGIELPKCVPVCGVPTEPIALQQRIFGGFPAKIQSFPWQVFFESPRAGGALIDEYWVLTAAHGRETLTHLCMWGPHL

SEQ ID NO: 12 - protein, 461 aa, Artificial sequence
  synthetic sequence
VPVWKEATTTLFCASDAKAYDTEAHNVWATHACVPTDPNPQEVELVNVTENFNMWKNNMVEQMHEDIISLWDQSLKPCVKLTPLCVTLNCTDLRNTTNTNNSTDNNNSKSEGTIKGGEMKNCSFNITTSIGDKMQKEYALLYKLDIEPIDNDSTSYRLISCNTSVITQACPKISFEPIPIHYCAPAGFAILKCNDKKFSGKGSCKNVSTVQCTHGIRPVVSTQLLLNGSLAEEEVVIRSEDFTDNAKTIIVHLKESVQINCTRPNNNTRKRIHIGPGRAFYTTKNIKGTIRQAHCNISRAKWNDTLRQIVSKLKEQFKNKTIVFNPSSGGDPEIVMHSFNCGGEFFYCNTSPLFNSIWNGNNTWNNTTGSNNNITLQCKIKQIINMWQKVGKAMYAPPIEGQIRCSSNITGLLLTRDGGEDTDTNDTEIFRPGGGDMRDNWRSELYKYKVVTIEPLGVAPT

SEQ ID NO: 13 - protein, 526 aa, Artificial sequence
  synthetic sequence
MGGAAARLGAVILFVVIVGLHGVRGKYALADASLKMADPNRFRGKDLPVLDQLLEVPVWKEATTTLFCASDAKAYDTEAHNVWATHACVPTDPNPQEVELVNVTENFNMWKNNMVEQMHEDIISLWDQSLKPCVKLTPLCVTLNCTDLRNTTNTNNSTDNNNSKSEGTIKGGEMKNCSFNITTSIGDKMQKEYALLYKLDIEPIDNDSTSYRLISCNTSVITQACPKISFEPIPIHYCAPAGFAILKCNDKKFSGKGSCKNVSTVQCTHGIRPVVSTQLLLNGSLAEEEVVIRSEDFTDNAKTIIVHLKESVQINCTRPNNNTRKRIHIGPGRAFYTTKNIKGTIRQAHCNISRAKWNDTLRQIVSKLKEQFKNKTIVFNPSSGGDPEIVMHSFNCGGEFFYCNTSPLFNSIWNGNNTWNNTTGSNNNITLQCKIKQIINMWQKVGKAMYAPPIEGQIRCSSNITGLLLTRDGGEDTDTNDTEIFRPGGGDMRDNWRSELYKYKVVTIEPLGVAPTKAKRRVVQRE

SEQ ID NO: 14 - DNA, 2085 bp, Artificial sequence
  synthetic sequence
atgggcaaatcaccagaggcatggtgcattgtcttgttttctgttttggcatcattttctgccgagcctaccatgcatggggagatcctgtcccctaactatcctcaggcgtaccccaatgagatcgagaaaacgtgggacatagaagtcccagaagggtttgggattcgcctctacttcacccatctggacatggagctgtcagagaactgcgaatatgactcggtgcagataatctcaggaggcgtcgaggaagggagactctgtgggcagaggaccagcaagaatgccaactcccccattgtggaagagtttcaaatgccatacaataaactccaggtgatctttaggtcagacttctccaacgaagagcggtttactggctttgctgcatattacgctgccgtagatataaatgaatgcacagattttacagatgtcccttgcagccacttctgcaataatttcattggtggttacttctgctcctgtcccccagaatacttcctccacgatgacatgaggaactgcggagtcaattgtagtgggaatgtattcactgccctgattggggagatttcaagccccaattatcccagtccataccccgagaactcaaggtgtgaataccagattttgctggaggaggggttccaagtggtggtgactatccggagagaagattttgatgtggaaccagctgactcggaggggaactgccaggacagtttactctttgctgcaaaaaatcaactatttggtccttactgtggcaatgggttccctgggccactaactattgaaacccacagtaacactcttgacattgtctttcaaacggacctaacagagcaaagaaaaggctggaagcttcgttaccatggagacccaatcccttgtcccaaggaaatcactgccaattctgtttgggtgcctgaaaaggcaaaatatgtgtttaaagatgtggtgaagatatcctgtgtggacggatttgaagttgtagagggaaatgttggctcagcattcttctattctacttgtcaaagcaatggacagtggagtaattccagactacaatgtcagcctgtggactgtggtattccggaacccattcagaatggtaaagttgacgatccagaaaacactgtgtttggctctgtcatccagtactcgtgcgaggagccatattactacatggaacatgaagaacacggcggggagtatcgctgcgctgctaatgggagctgggtgaatgacgaactgggcatagagctcccaaaatgtgttccagtctgtggggtacccactgagcccattgcattacagcagaggatatttggaggattccctgcaaagatccagagttttccttggcaagtcttctttgagtccccacgggccggtggggctcttattgacgagtactgggtgttgacagccgcttttgtggagggaaactctgacccatctatgtatgtggggaccacatttgtgagaatggaacatctggcgaatgcccagaggctcaccgctgaacgtgtgattattcatccaggctggaagccagcggatgacctagaaacacggacaaattttgacaatgacattgcactggtgcagctgaaagaccccgtgaaaatggggcccactgtctcccccatctgcctgccaggtacctcctcagagtacaacccctcaaagaatgacctgggactgatctcagggtggggccgaacagagaagagaaatattgttccccaactcaaaggggcaaagttacctgtgacctctttagagaagtgccaacaggtgaaaggggagaactccaaagtgagggcggatgactacgttttcaccagcaacatgatctgtgctggagagaaaggtgttgatagctgtcagggggacagtggtggggcttttgctttgcaggtccccaatgtaaaggaccccaaattctatgtggcaggcctagtgtcctgggggaaaaagtgtgggacctatggaatctacacaaaggtaaagaactacatggattggatcgtgaagacgatgcaggagaatagtgtccccagtaaggactaa

SEQ ID NO: 15 - protein, 684 aa, Artificial sequence
  synthetic sequence
MRVKGIRRNYQHWWGWGTMLLGLLMICSATEKLWVTVYYGVPVWKEATTTLFCASDAKAYDTEAHNVWATHACVPTDPNPQEVELVNVTENFNMWKNNMVEQMHEDIISLWDQSLKPCVKLTPLCVTLNCTDLRNTTNTNNSTDNNNSKSEGTIKGGEMKNCSFNITTSIGDKMQKEYALLYKLDIEPIDNDSTSYRLISCNTSVITQACPKISFEPIPIHYCAPAGFAILKCNDKKFSGKGSCKNVSTVQCTHGIRPVVSTQLLLNGSLAEEEVVIRSEDFTDNAKTIIVHLKESVQINCTRPNNNTRKRIHIGPGRAFYTTKNIKGTIRQAHCNISRAKWNDTLRQIVSKLKEQFKNKTIVFNPSSGGDPEIVMHSFNCGGEFFYCNTSPLFNSIWNGNNTWNNTTGSNNNITLQCKIKQIINMWQKVGKAMYAPPIEGQIRCSSNITGLLLTRDGGEDTDTNDTEIFRPGGGDMRDNWRSELYKYKVVTIEPLGVAPTKAKRRVVQREKRAAIGALFLGFLGAAGSTMGAASVTLTVQARLLLSGIVQQQNNLLRAIEAQQHMLQLTVWGIKQLQARVLAVERYLKDQQLLGFWGCSGKLICTTTVPWNASWSNKSLDDIWNNMTWMQWEREIDNYTSLIYSLLEKSQTQQEKNEQELLELDKWASLWNWFDITNWLWYIK

SEQ ID NO: 16 - protein, 694 aa, Artificial sequence
  synthetic sequence
MGKSPEAWCIVLFSVLASFSAEPTMHGEILSPNYPQAYPNEIEKTWDIEVPEGFGIRLYFTHLDMELSENCEYDSVQIISGGVEEGRLCGQRTSKNANSPIVEEFQMPYNKLQVIFRSDFSNEERFTGFAAYYAAVDINECTDFTDVPCSHFCNNFIGGYFCSCPPEYFLHDDMRNCGVNCSGNVFTALIGEISSPNYPSPYPENSRCEYQILLEEGFQVVVTIRREDFDVEPADSEGNCQDSLLFAAKNQLFGPYCGNGFPGPLTIETHSNTLDIVFQTDLTEQRKGWKLRYHGDPIPCPKEITANSVWVPEKAKYVFKDVVKISCVDGFEVVEGNVGSAFFYSTCQSNGQWSNSRLQCQPVDCGIPEPIQNGKVDDPENTVFGSVIQYSCEEPYYYMEHEEHGGEYRCAANGSWVNDELGIELPKCVPVCGVPTEPIALQQRIFGGFPAKIQSFPWQVFFESPRAGGALIDEYWVLTAAFVEGNSDPSMYVGTTFVRMEHLANAQRLTAERVIIHPGWKPADDLETRTNFDNDIALVQLKDPVKMGPTVSPICLPGTSSEYNPSKNDLGLISGWGRTEKRNIVPQLKGAKLPVTSLEKCQQVKGENSKVRADDYVFTSNMICAGEKGVDSCQGDSGGAFALQVPNVKDPKFYVAGLVSWGKKCGTYGIYTKVKNYMDWIVKTMQENSVPSKD

SEQ ID NO: 17 - DNA, 20 bp, Artificial sequence
  synthetic sequence
gataatctcaggaggcgtcg

SEQ ID NO: 18 - DNA, 20 bp, Artificial sequence
  synthetic sequence
gccagtaaaccgctcttcgt

SEQ ID NO: 19 - DNA, 20 bp, Artificial sequence
  synthetic sequence
gttgacagccgctcatgttg

SEQ ID NO: 20 - protein, 680 aa, Artificial sequence
  synthetic sequence
MRVTEIRKSYQHWWRWGIMLLGILMICNAEEKLWVTVYYGVPVWKEATTTLFCASDAKAYDTEVHNVWATHACVPTDPNPQEVALENVTENFNMWKNNMVEQMHEDIISLWDQSLKPCVKLTPLCVTLNCTDLRNATSRNVTNTTSSSRGMVGGGEMKNCSFNITTGIRGKVQKEYALFYELDIVPIDNKIDRYRLISCNTSVITQACPKVSFEPIPIHYCAPAGFAILKCKDKKFNGKGPCSNVSTVQCTHGIRPVVSTQLLLNGSLAEEEVVIRSENFTNNAKTIIVQLNESVEINCTRPNNNTRKSINIGPGRAFYTTGEIIGDIRQAHCNLSRAKWNDTLNKIVIKLREQFGNKTIVFKHSSGGDPEIVTHSFNCGGEFFYCNSTQLFNSTWNVTEESNNTVENNTITLPCRIKQIINMWQEVGRAMYAPPIRGQIRCSSNITGLLLTRDGGPEDNKTEVFRPGGGDMRDNWRSELYKYKVVKIEPLGVAPTKAKRRVVQREKRAVGIGAVFLGFLGAAGSTMGAASMTLTVQARLLLSGIVQQQNNLLRAIEAQQHLLQLTVWGIKQLQARVLAVERYLRDQQLLGIWGCSGKLICTTAVPWNASWSNKSLNKIWDNMTWMEWDREINNYTSIIYSLIEESQNQQEKNEQELLELDKWASLWNWFDITKWLWYIK

SEQ ID NO: 21 - DNA, 23 bp, Artificial sequence
  synthetic sequence
gccagcattgattcctgcatctc

SEQ ID NO: 22 - protein, 453 aa, Artificial sequence
  synthetic sequence
VPVWKEAKTTLFCASEAKGYEKEVHNVWATHACVPTDPSPHELVLENVTENFNMWENDMVDQMHEDIISLWDQSLKPCVKLTPLCVTLNCTNVTGTNVTGNDMKGEMTNCSFNATTEIKDRKKNVYALFYKLDVVQLEGNSSNSTYSTYRLINCNTSVITQACPKVSFDPIPIHYCAPAGYAILKCNNKTFNGTGPCNNVSTVQCTHGIKPVVSTQLLLNGSLAEKEIVIRSKNLTDNVKTIIVHLNESVEITCIRPGNNTRKSIRIGPGQAFYATGDIIGNIRQAHCNISEDKWNKTLQMVGEKLGKLFPNKTIKEPASGGDLEITTHSFNCRGEFFYCNTTKLFNSTYRPNANANSSSSNNTITLQCKIKQIINMWQEVGRAMYAPPIAGNITCTSNITGLLLVRDGGNNSTEEEIFRPGGGNMKDNWRSELYKYKVVEIKPLGVAPTGAK

SEQ ID NO: 23 - protein, 531 aa, Artificial sequence
  synthetic sequence
MGGAAARLGAVILFVVIVGLHGVRGKYALADASLKMADPNRFRGKDLPVLDQLLEVPVWKEAKTTLFCASEAKGYEKEVHNVWATHACVPTDPSPHELVLENVTENFNMWENDMVDQMHEDIISLWDQSLKPCVKLTPLCVTLNCTNVTGTNVTGNDMKGEMTNCSFNATTEIKDRKKNVYALFYKLDVVQLEGNSSNSTYSTYRLINCNTSVITQACPKVSFDPIPIHYCAPAGYAILKCNNKTFNGTGPCNNVSTVQCTHGIKPVVSTQLLLNGSLAEKEIVIRSKNLTDNVKTIIVHLNESVEITCIRPGNNTRKSIRIGPGQAFYATGDIIGNIRQAHCNISEDKWNKTLQMVGEKLGKLFPNKTIKEPASGGDLEITTHSFNCRGEFFYCNTTKLFNSTYRPNANANSSSSNNTITLQCKIKQIINMWQEVGRAMYAPPIAGNITCTSNITGLLLVRDGGNNSTEEEIFRPGGGNMKDNWRSELYKYKVVEIKPLGVAPTGAKRRVVEREKRAVGIGAVFLGFLGA

SEQ ID NO: 24 - DNA, 23 bp, Artificial sequence
  synthetic sequence
cccattttcacggggtctttcag

SEQ ID NO: 25 - protein, 457 aa, Artificial sequence
  synthetic sequence
VPVWKEATTTLFCASDAKAYDTEVRNVWATHACVPADPNPQEMVLENVTENFNMWKNEMVNQMQEDVISLWDQSLKPCVKLTPLCVTLECRNVSSNSNGAHNETYHESMKEMKNCSFNATTVVRDRKQTVYALFYRLNIVPLTKKNSSENSSEYYRLINCNTSAITQACPKVTFDPIPIHYCTPAGYAILKCNDKIFNGTGPCHNVSTVQCTHGIKPVVSTQLLLNGSLAEGEIIIRSENLTNNVKTIIVHLNQSVEIVCTRPGNNTRKSIRIGPGQTFYATGDIIGDIRQAHCNISEDKWNETLQRVSKKLAEHFQNKTIKFASSSGGDLEITTHSFNCRGEFFYCNTSGLFNGTYTPNGTKSNSSSIITIPCRIKQIINMWQEVGRAMYAPPIEGNITCKSNITGLLLVRDGGTEPNDTETFRPGGGDMRNNWRSELYKYKVVEIKPLGVAPTTA

SEQ ID NO: 26 - DNA, 23 bp, Artificial sequence
  synthetic sequence
gttgacagccgctcatgttgtgg

SEQ ID NO: 27 - protein, 856 aa, HIV
MRVKEKYQHLWRWGWRWGTMLLGMLMICSATEKLWVTVYYGVPVWKEATTTLFCASDAKAYDTEVHNVWATHACVPTDPNPQEVVLVNVTENFNMWKNDMVEQMHEDIISLWDQSLKPCVKLTPLCVSLKCTDLKNDTNTNSSSGRMIMEKGEIKNCSFNISTSIRGKVQKEYAFFYKLDIIPIDNDTTSYKLTSCNTSVITQACPKVSFEPIPIHYCAPAGFAILKCNNKTFNGTGPCTNVSTVQCTHGIRPVVSTQLLLNGSLAEEEVVIRSVNFTDNAKTIIVQLNTSVEINCTRPNNNTRKRIRIQRGPGRAFVTIGKIGNMRQAHCNISRAKWNNTLKQIASKLREQFGNNKTIIFKQSSGGDPEIVTHSFNCGGEFFYCNSTQLFNSTWFNSTWSTEGSNNTEGSDTITLPCRIKQIINMWQKVGKAMYAPPISGQIRCSSNITGLLLTRDGGNSNNESEIFRPGGGDMRDNWRSELYKYKVVKIEPLGVAPTKAKRRVVQREKRAVGIGALFLGFLGAAGSTMGAASMTLTVQARQLLSGIVQQQNNLLRAIEAQQHLLQLTVWGIKQLQARILAVERYLKDQQLLGIWGCSGKLICTTAVPWNASWSNKSLEQIWNHTTWMEWDREINNYTSLIHSLIEESQNQQEKNEQELLELDKWASLWNWFNITNWLWYIKLFIMIVGGLVGLRIVFAVLSIVNRVRQGYSPLSFQTHLPTPRGPDRPEGIEEEGGERDRDRSIRLVNGSLALIWDDLRSLCLFSYHRLRDLLLIVTRIVELLGRRGWEALKYWWNLLQYWSQELKNSAVSLLNATAIAVAEGTDRVIEVVQGACRAIRHIPRRIRQGLERILL

SEQ ID NO: 28 - protein, 504 aa, Artificial sequence
  synthetic sequence
MPMGSLQPLATLYLLGMLVASVLAAENLWVTVYYGVPVWKDAETTLFCASDAKAYETEKHNVWATHACVPTDPNPQEIHLENVTEEFNMWKNNMVEQMHTDIISAWDQSLKPCVKLTPLCVTLQCTNVTNNITDDMRGELKNCSFNMTTELRDKKQKVYSLFYRLDVVQINENQGNRSNNSNKEYRLINCNTSAITQACPKVSFEPIPIHYCAPAGFAILKCKDKKFNGTGPCPSVSTVQCTHGIKPVVSTQLLLNGSLAEEEVMIRSENITNNAKNILVQFNTPVQINCTRPNNNTRKSIRIGPGQAFYATGDIIGDIRQAHCNVSKATWNETLGKVVKQLRKHFGNNTIIRFANSSGGDLEVTTHSFNCGGEFFYCNTSGLFNSTWISNTSVQGSNSTGSNDSITLPCRIKQIINMWQRIGQAMYAPPIQGVIRCVSNITGLILTRDGGSTNSTTETFRPGGGDMRDNWRSELYKYKVVKIEPLGVAPTRAKSSVVGSEKSG

SEQ ID NO: 29 - DNA, 23 bp, Artificial sequence
  synthetic sequence
gttgacagccgctcatgttgtgg

SEQ ID NO: 30 - DNA, 23 bp, Artificial sequence
  synthetic sequence
gttgacagccgctcatgttgtgg

SEQ ID NO: 31 - protein, 35 aa, Artificial sequence
  synthetic sequence
CTRPNNNTRKSIRIQRGPGRAFVIGKIGNMRQAHC

SEQ ID NO: 32 - protein, 515 aa, Artificial sequence
  synthetic sequence
MRVMGTQKNCQQWWIWGILGFWMLMICNTKDLWVTVYYGVPVWREAKTTLFCASDAKAYETEVHNVWATHACVPTDPNPQEIVLGNVTENFNMWKNDMADQMHEDIISLWDQSLKPCVKLTPLCVTLNCTETNVTGNRTVIGNTNDTNIANATYKYEEMKNCSFNVTTELRNKKHKEYALFYRLDIVPLNENGDNSKYRLINCNTSAITQACPKVSFDPIPIHYCAPAGYAILKCNNKTFNGTGPCYNVSTVQCTHGIKPVVSTQLLLNGSLAEEGMIIRSENLTENTKTIIVHLNESVEINCTRPNNNTRKSVRIGPGQAFYATNDVIGDIRQAHCNISTDRWNKTLQQVMKKLGEHFPNKTIQFKPHAGGDIEITMHSFNCRGEFFYCNTSNLFNSTYHSNNGTYKYNGNSSSPITLQCKIKQIVRMWQGVGQAMYAPPIAGNITCRSNITGILLTRDGGFNTTNNTETFRPGGGDMRDNWRSELYKYKVVEIKPLGIAPTKAKRRVVQREKR

SEQ ID NO: 33 - protein, 8 aa, Artificial sequence
  synthetic sequence
  misc_feature (1)..(8): Xaa can be any naturally occurring amino acid
XXXXXXXX

SEQ ID NO: 34 - protein, 687 aa, Artificial sequence
  synthetic sequence
MRVMGTQKNCQQWWIWGILGFWMLMICNTKDLWVTVYYGVPVWREAKTTLFCASDAKAYETEVHNVWATHACVPTDPNPQEIVLGNVTENFNMWKNDMADQMHEDIISLWDQSLKPCVKLTPLCVTLNCTETNVTGNRTVIGNTNDTNIANATYKYEEMKNCSFNVTTELRNKKHKEYALFYRLDIVPLNENGDNSKYRLINCNTSAITQACPKVSFDPIPIHYCAPAGYAILKCNNKTFNGTGPCYNVSTVQCTHGIKPVVSTQLLLNGSLAEEGMIIRSENLTENTKTIIVHLNESVEINCTRPNNNTRKSVRIGPGQAFYATNDVIGDIRQAHCNISTDRWNKTLQQVMKKLGEHFPNKTIQFKPHAGGDIEITMHSFNCRGEFFYCNTSNLFNSTYHSNNGTYKYNGNSSSPITLQCKIKQIVRMWQGVGQAMYAPPIAGNITCRSNITGILLTRDGGFNTTNNTETFRPGGGDMRDNWRSELYKYKVVEIKPLGIAPTKAKRRVVQREKRAVGIGAVFLGFLGAAGSTMGAASITLTVQARQLLSGIVQQQSNLLKAIEAQQHMLQLTVWGIKQLQARVLAIERYLKDQQLLGIWGCSGRLICTTAVPWNSSWSNKSEADIWDNMTWMQWDREINNYTEAIFRLLEDSQNQQEKNEKDLLELDKWNSLWNWFNISNWLWYIK

SEQ ID NO: 35 - protein, 8 aa, Artificial sequence
  synthetic sequence
  misc_feature (1)..(8): Xaa can be any naturally occurring amino acid
XXXXXXXX

SEQ ID NO: 36 - protein, 488 aa, Artificial sequence
  synthetic sequence
MRVRGIWKNWPQWLIWSILGFWIGNMEGSWVTVYYGVPVWKEAKTTLFCASDAKAYEKEVHNVWATHACVPTDPNPQEMVLANVTENFNMWKNDMVEQMHEDIISLWDESLKPCVKLTPLCVTLNCTNVKGNESDTSEVMKNCSFKATTELKDKKHKVHALFYKLDVVPLNGNSSSSGEYRLINCNTSAITQACPKVSFDPIPLHYCAPAGFAILKCNNKTFNGTGPCRNVSTVQCTHGIKPVVSTQLLLNGSLAEEEIIIRSENLTNNAKTIIVHLNESVNIVCTRPNNNTRKSIRIGPGQTFYATGDIIGNIRQAHCNINESKWNNTLQKVGEELAKHFPSKTIKFEPSSGGDLEITTHSFNCRGEFFYCNTSDLFNGTYRNGTYNHTGRSSNGTITLQCKIKQIINMWQEVGRAIYAPPIEGEITCNSNITGLLLLRDGGQSNETNDTETFRPGGGDMRDNWRSELYKYKVVEIKPLGVAPTEAK

SEQ ID NO: 37 - protein, 8 aa, Artificial sequence
  synthetic sequence
  misc_feature (1)..(8): Xaa can be any naturally occurring amino acid
XXXXXXXX

SEQ ID NO: 38 - protein, 669 aa, Artificial sequence
  synthetic sequence
MRVRGIWKNWPQWLIWSILGFWIGNMEGSWVTVYYGVPVWKEAKTTLFCASDAKAYEKEVHNVWATHACVPTDPNPQEMVLANVTENFNMWKNDMVEQMHEDIISLWDESLKPCVKLTPLCVTLNCTNVKGNESDTSEVMKNCSFKATTELKDKKHKVHALFYKLDVVPLNGNSSSSGEYRLINCNTSAITQACPKVSFDPIPLHYCAPAGFAILKCNNKTFNGTGPCRNVSTVQCTHGIKPVVSTQLLLNGSLAEEEIIIRSENLTNNAKTIIVHLNESVNIVCTRPNNNTRKSIRIGPGQTFYATGDIIGNIRQAHCNINESKWNNTLQKVGEELAKHFPSKTIKFEPSSGGDLEITTHSFNCRGEFFYCNTSDLFNGTYRNGTYNHTGRSSNGTITLQCKIKQIINMWQEVGRAIYAPPIEGEITCNSNITGLLLLRDGGQSNETNDTETFRPGGGDMRDNWRSELYKYKVVEIKPLGVAPTEAKRRVVEREKRAVGIGAVFLGFLGAAGSTMGAASMTLTVQARQLLSGIVQQQSNLLRAIEAQQHMLQLTVWGIKQLQARVLAIERYLKDQQLLGMWGCSGKLICTTAVPWNSSWSNKSQNEIWGNMTWMQWDREINNYTNTIYRLLEDSQNQQEKNEKDLLALDSWKNLWNWFDISKWLWYIK

SEQ ID NO: 39 - protein, 8 aa, Artificial sequence
  synthetic sequence
  misc_feature (1)..(8): Xaa can be any naturally occurring amino acid
XXXXXXXX

SEQ ID NO: 40 - protein, 492 aa, Artificial sequence
  synthetic sequence
MRVRGILRNWPQWWIWSILGFWMLIICRVMGNLWVTVYYGVPVWKEAKATLFCASDARAYEKEVHNVWATHACVPTDPNPQEIYLGNVTENFNMWKNDMVDQMHEDIISLWDQSLKPCVKLTPLCVTLRCTNATINGSLTEEVKNCSFNITTELRDKKQKAYALFYRPDVVPLNKNSPSGNSSEYILINCNTSTITQACPKVSFDPIPIHYCAPAGYAILKCNNKTFNGTGPCNNVSTVQCTHGIKPVVSTQLLLNGSLAEEDIIIKSENLTNNIKTIIVHLNKSVEIVCRRPNNNTRKSIRIGPGQAFYATNDIIGDIRQAHCNINNSTWNRTLEQIKKKLREHFLNRTIEFEPPSGGDLEVTTHSFNCGGEFFYCNTTRLFKWSSNVTNDTITIPCRIKQFINMWQGAGRAMYAPPIEGNITCNSSITGLLLTRDGGKTDRNDTEIFRPGGGNMKDNWRNELYKYKVVEIKPLGVAPTEARRRVVEREKR

SEQ ID NO: 41 - protein, 8 aa, Artificial sequence
  synthetic sequence
  misc_feature (1)..(8): Xaa can be any naturally occurring amino acid
XXXXXXXX

SEQ ID NO: 42 - protein, 664 aa, Artificial sequence
  synthetic sequence
MRVRGILRNWPQWWIWSILGFWMLIICRVMGNLWVTVYYGVPVWKEAKATLFCASDARAYEKEVHNVWATHACVPTDPNPQEIYLGNVTENFNMWKNDMVDQMHEDIISLWDQSLKPCVKLTPLCVTLRCTNATINGSLTEEVKNCSFNITTELRDKKQKAYALFYRPDVVPLNKNSPSGNSSEYILINCNTSTITQACPKVSFDPIPIHYCAPAGYAILKCNNKTFNGTGPCNNVSTVQCTHGIKPVVSTQLLLNGSLAEEDIIIKSENLTNNIKTIIVHLNKSVEIVCRRPNNNTRKSIRIGPGQAFYATNDIIGDIRQAHCNINNSTWNRTLEQIKKKLREHFLNRTIEFEPPSGGDLEVTTHSFNCGGEFFYCNTTRLFKWSSNVTNDTITIPCRIKQFINMWQGAGRAMYAPPIEGNITCNSSITGLLLTRDGGKTDRNDTEIFRPGGGNMKDNWRNELYKYKVVEIKPLGVAPTEARRRVVEREKRAVGIGAVLLGFLGAAGSTMGAASITLTVQARQLLSGIVQQQSNLLRAIEAQQHMLQLTVWGIKQLQTRVLAIERYLKDQQLLGLWGCSGKLICTTNVPWNSSWSNKSQTDIWDNMTWIQWDREISNYSNTIYKLLEGSQNQQEQNEKDLLALDSWNNLWNWFNITNWLWYIK

SEQ ID NO: 43 - protein, 8 aa, Artificial sequence
  synthetic sequence
  misc_feature (1)..(8): Xaa can be any naturally occurring amino acid
XXXXXXXX

SEQ ID NO: 44 - protein, 25 aa, Artificial sequence
  synthetic sequence
MGGAAARLGAVILFVVIVGLHGVRG

SEQ ID NO: 45 - protein, 21 aa, Artificial sequence
  synthetic sequence
MAYPAVIVLVCGLFWVPATQG

SEQ ID NO: 46 - protein, 27 aa, Artificial sequence
  synthetic sequence
MAPSSPRPALPALLVLLGALFPGPGNA

SEQ ID NO: 47 - protein, 36 aa, Artificial sequence
  synthetic sequence
MDAMKRGLCCVLLLCGAVFVSPSQEIHARFRRGARW

SEQ ID NO: 48 - protein, 27 aa, Artificial sequence
  synthetic sequence
KYALADASLKMADPNRFRGKDLPVLDQ

SEQ ID NO: 49 - protein, 27 aa, Artificial sequence
  synthetic sequence
YVRADPSLSMVNPNRFRGGHLPPLVQQ

SEQ ID NO: 50 - protein, 11 aa, Artificial sequence
  synthetic sequence
TDNLWVTVYYG

SEQ ID NO: 51 - protein, 6 aa, Artificial sequence
  synthetic sequence
HHHHHH

SEQ ID NO: 52 - protein, 15 aa, Artificial sequence
  synthetic sequence
GLNDIFEAQKIEWHE

SEQ ID NO: 53 - protein, 8 aa, Artificial sequence
  synthetic sequence
WSHPQFEK

SEQ ID NO: 54 - protein, 16 aa, Artificial sequence
  synthetic sequence
HHHHHHSSWSHPQFEK

SEQ ID NO: 55 - protein, 24 aa, Artificial sequence
  synthetic sequence
HHHHHHSSWSHPQFEKSSHHHHHH

SEQ ID NO: 56 - protein, 23 aa, Artificial sequence
  synthetic sequence
HHHHHHWSHPQFEKHHHHHHQSG

SEQ ID NO: 57 - protein, 8 aa, Artificial sequence
  synthetic sequence
KRRVVQRE

SEQ ID NO: 58 - protein, 23 aa, Artificial sequence
  synthetic sequence
RRVVEREKRAVGIGAVFLGFLGA